European Patent Application EP 4 502 165 A1, published February 5, 2025. Title: Novel recombinant vectors and uses thereof. Applicant: Cell&Brain Co., Ltd. The sequence listing filed with the application follows.

SEQUENCE LISTING (53 sequences)

SEQ ID NO: 1 - DNA, 170 bp, Mason-Pfizer monkey virus
  source 1..170: mol_type = genomic DNA
ccacctcccctgcgagctaagctggacagccaatgacgggtaagagagtgacatttttcactaacctaagacaggagggccgtcagagctactgcctaatccaaagacgggtaaaagtgataaaaatgtatcactccaacctaagacaggcgcagcttccgagggatttg

SEQ ID NO: 2 - DNA, 1295 bp, synthetic construct
  source 1..1295: mol_type = other DNA
ctgtaggaaaaagaagaaggcatgaacatggttagcagaggctctagagccgccggtcacacgccagaagccgaaccccgccctgccccgtcccccccgaaggcagccgtccccccgcggacagccccgaggctggagagggagaaggggacggcggcgcggcgacgcacgaaggccctccccgcccatttccttcctgccggcgccgcaccgcttcgccccgcgcccgctagagggggtgcggcggcgcctcccagatttcggctccgcacagatttgggacaaaggaagtccctgcgccctctcgcacgattaccataaaaggcaatggctgcggctcgccgcgcctcgacagccgccggcgctccgggggccgccgcgcccctcccccgagccctccccggcccgaggcggccccgccccgcccggcacccccacctgccgccaccccccgcccggcacggcgagccccgcgccacgccccgtacggagccccgcacccgaagccgggccgtgctcagcaactcggggaggggggtgcagggggggttgcagcccgaccgacgcgcccacaccccctgctcacccccccacgcacacaccccgcacgcagcctttgttcccctcgcagccccccccgcaccgcggggcaccgcccccggccgcgctcccctcgcgcacactgcggagcgcacaaagccccgcgccgcgcccgcagcgctcacagccgccgggcagcgcggagccgcacgcggcgctccccacgcacacacacacgcacgcaccccccgagccgctccccccgcacaaagggccctcccggagcccctcaaggctttcacgcagccacagaaaagaaacaagccgtcattaaaccaagcgctaattacagcccggaggagaagggccgtcccgcccgctcacctgtgggagtaacgcggtcagtcagagccggggcgggcggcgcgaggcggcggcggagcggggcacggggcgaaggcagcgcgcagcgactcccgcccgccgcgcgcttcgctttttatagggccgccgccgccgccgcctcgccataaaaggaaactttcggagcgcgccgctctgattggctgccgccgcacctctccgcctcgccccgccccgcccctcgccccgccccgccccgcctggcgcgcgcccccccccccgccccgcccccatcgctgcacaaaataattaaaaaataaataaatacaaaattgggggtggggaggggggggagatggggagagtgaagcagaacgtggggctcacctcga

SEQ ID NO: 3 - DNA, 431 bp, synthetic construct
  source 1..431: mol_type = other DNA
catggtaatagcgatgactaatacgtagatgtactgccaagtaggaaagtcccataaggtcatgtactgggcataatgccaggcgggccatttaccgtcattgacgtcaatagggggcgtacttggcatatgatacacttgatgtactgccaagtgggcagtttaccgtaaatactccacccattgacgtcaatggaaagtccctattggcgttactatgggaacatacgtcattattgacgtcaatgggcgggggtcgttgggcggtcagccaggcgggccatttaccgtaagttatgtaacgcggaactccatatatgggctatgaactaatgaccccgtaattgattactattaataactagtcaataatcaatgtcgacatcgtcgagggtaggcgtgtacggtgggaggcctatataagcagagct

SEQ ID NO: 4 - DNA, 500 bp, synthetic construct
  source 1..500: mol_type = other DNA
gggtaggggaggcgcttttcccaaggcagtctggagcatgcgctttagcagccccgctgggcacttggcgctacacaagtggcctctggcctcgcacacattccacatccaccggtaggcgccaaccggctccgttctttggtggccccttcgcgccaccttctactcctcccctagtcaggaagttcccccccgccccgcagctcgcgtcgtgcaggacgtgacaaatggaagtagcacgtctcactagtctcgtgcagatggacagcaccgctgagcaatggaagcgggtaggcctttggggcagcggccaatagcagctttgctccttcgctttctgggctcagaggctgggaaggggtgggtccgggggcgggctcaggggcgggctcaggggcggggcgggcgcccgaaggtcctccggaggcccggcattctgcacgcttcaaaagcgcacgtctgccgcgctgttctcctcttcctcatctccgggcctttcg

SEQ ID NO: 5 - DNA, 298 bp, synthetic construct
  source 1..298: mol_type = other DNA
ggtgtggaaagtccccaggctccccagcaggcagaagtatgcaaagcatgcatctcaattagtcagcaaccaggtgtggaaagtccccaggctccccagcaggcagaagtatgcaaagcatgcatctcaattagtcagcaaccatagtcccgcccctaactccgcccatcccgcccctaactccgcccagttccgcccattctccgccccatggctgactaattttttttatttatgcagaggccgaggccgcctcggcctctgagctattccagaagtagtgaggaggcttttttgg

SEQ ID NO: 6 - DNA, 2187 bp, Homo sapiens
  source 1..2187: mol_type = genomic DNA
ctatgactgtggtaccttatatgttaaaataattttgtgtatccattttgcataatatgctactcggacaaaaataccaggacgatttggaatggcacatccacgaccaggaacaatgacaccaagaaccattctcattttatgttgctcacaaacaagtgggccaccataatccccctcacatggtcctgatccaatcttttcagccccagcacatatttcagactcattcagagtcaccttccctcgatgatgctggctgcatttctcatttcccattatatagagatgtgccactcgtaataggccatcatagttgatcaatccagtgtagccccagccataaacactgcaactggtcttttcaggaattgtgcatccataattaggtaaatcaatcgtactaacaaaatcatccaggacagcaggcctggcaagcttcattaaaaccagatctgatccttcagggccatataccagctgggaaacattgagaacctgtttgcatttctcatctcctcttccgtggacatcatgaattccaagccaagcttcataatctttcaagtctcgagaagggaaacactgtcgtgcagtaagaacccaactctcctttatcaatgatcctccgcagatatgtttatttctgtatctcaaactaaccatccatcctatgtttgttcgtgttggaatcccatttacaactcgcaattgtttcgttttggcacaagatattacgggatggtctaaattgactattgtaggtgtggtatcaccttcacaacgagaaatagggcaataatcccaaggaatgagtggatttcccgtgtagcaccagggtccatgagcatcatcatctggatttcggcagtaattctcattcagcttacttgcatctggttcccagaagatatgacgatgtaagtcttccatgttcttgtcccacattgaacatgttagtccagatcttgtttgggataagttgcccatataatttttgccattcccacgataacaatcttgtccatgtgacatatcacagtttggaatttgggagcagtagccaactcggatgtttggatcagtggtaaaacaccagggtgattcagacccatctggatttcggcagtaattttctcgtaggtccttgcacttgaaattttcaggagtcatgtcatgctcgtgaggatactgagaatcccaacgctgacatggaattccattccaaatggtattgacagtgcccctgtagccttctccttgaccttggatgcattcagttgtttccaaaggaacatcagtgtcattcatagtattgtcagcgcatgttttaattgcacagtactcccagcgggtgtgagggtcaagagtatagcaccatggcctcggctggccatcgggattgcggcaataattatcatcaaagcccttgtcgggatatctttcaggcaagaatttgtgccggtgtggtgtctgatgatcccagcgctgacaaatcttgcctgattctgtatgatccatgagacctcgataactctccccattgcaggtcatgcattcaacttctgaacactgaggaatgtcacagacttcgtagcgtacctctggattgcttgtgaaacaccagggtcccccttcttcccctcgaggatttcgacagtagttttcctgtaggtctttaccccgatagctcgaaggcaaaaagctgtgttcgtgtggtatcatggaactccagggctgacatttgatgccactcttagtgatagatactgttcccttgtagctgcgtcctttaccaatgatgcagtttctaatgtagtctttgttttcatagaggtcaaattcatggccaaattcttttttcactccacttgacatgctattgaaggggaaccagaggcattgttttcttgctttatcaaaaacaaaagccttgcaagtgaatggaagtcctttattcctagtacatctattagcacattggtctgcagtattcacttttttggtttttatcttcagtgctggatctattttgattagggtagtctttgctgattttttgaattcatgaattgtatttcttcttttcctttgtccctctgcataggggatggcgatggggagcaggaggagatgcaggaggacatgctgcagcagcagggctggcaggagtttggtcacccacat

SEQ ID NO: 7 - DNA, 714 bp, Homo sapiens
  source 1..714: mol_type = genomic DNA
atgccagcccgccttgagacctgcatctccgacctcgactgcgccagcagcagcggcagtgacctatccggcttcctcaccgacgaggaagactgtgccagactccaacaggcagcctccgcttcggggccgcccgcgccggcccgcaggggcgcgcccaatatctcccgggcgtctgaggttccaggggcacaggacgacgagcaggagaggcggcggcgccgcggccggacgcgggtccgctccgaggcgctgctgcactcgctgcgcaggagccggcgcgtcaaggccaacgatcgcgagcgcaaccgcatgcacaacttgaacgcggccctggacgcactgcgcagcgtgctgccctcgttccccgacgacaccaagctcaccaaaatcgagacgctgcgcttcgcctacaactacatctgggctctggccgagacactgcgcctggcggatcaagggctgcccggaggcggtgcccgggagcgcctcctgccgccgcagtgcgtcccctgcctgcccggtcccccaagccccgccagcgacgcggagtcctggggctcaggtgccgccgccgcctccccgctctctgaccccagtagcccagccgcctccgaagacttcacctaccgccccggcgaccctgttttctccttcccaagcctgcccaaagacttgctccacacaacgccctgtttcattccttaccactag

SEQ ID NO: 8 - DNA, 738 bp, synthetic construct
  source 1..738: mol_type = other DNA
gattacaaggatgacgacgataagatgccagcccgccttgagacctgcatctccgacctcgactgcgccagcagcagcggcagtgacctatccggcttcctcaccgacgaggaagactgtgccagactccaacaggcagcctccgcttcggggccgcccgcgccggcccgcaggggcgcgcccaatatctcccgggcgtctgaggttccaggggcacaggacgacgagcaggagaggcggcggcgccgcggccggacgcgggtccgctccgaggcgctgctgcactcgctgcgcaggagccggcgcgtcaaggccaacgatcgcgagcgcaaccgcatgcacaacttgaacgcggccctggacgcactgcgcagcgtgctgccctcgttccccgacgacaccaagctcaccaaaatcgagacgctgcgcttcgcctacaactacatctgggctctggccgagacactgcgcctggcggatcaagggctgcccggaggcggtgcccgggagcgcctcctgccgccgcagtgcgtcccctgcctgcccggtcccccaagccccgccagcgacgcggagtcctggggctcaggtgccgccgccgcctccccgctctctgaccccagtagcccagccgcctccgaagacttcacctaccgccccggcgaccctgttttctccttcccaagcctgcccaaagacttgctccacacaacgccctgtttcattccttaccactag

SEQ ID NO: 9 - DNA, 1131 bp, Human alphaherpesvirus 1
  source 1..1131: mol_type = genomic DNA
atggcttcgtacccctgccatcaacacgcgtctgcgttcgaccaggctgcgcgttctcgcggccatagcaaccgacgtacggcgttgcgccctcgccggcagcaagaagccacggaagtccgcctggagcagaaaatgcccacgctactgcgggtttatatagacggtcctcacgggatggggaaaaccaccaccacgcaactgctggtggccctgggttcgcgcgacgatatcgtctacgtacccgagccgatgacttactggcaggtgctgggggcttccgagacaatcgcgaacatctacaccacacaacaccgcctcgaccagggtgagatatcggccggggacgcggcggtggtaatgacaagcgcccagataacaatgggcatgccttatgccgtgaccgacgccgttctggctcctcatatcgggggggaggctgggagctcacatgccccgcccccggccctcaccctcatcttcgaccgccatcccatcgccgccctcctgtgctacccggccgcgcgataccttatgggcagcatgaccccccaggccgtgctggcgttcgtggccctcatcccgccgaccttgcccggcacaaacatcgtgttgggggcccttccggaggacagacacatcgaccgcctggccaaacgccagcgccccggcgagcggcttgacctggctatgctggccgcgattcgccgcgtttacgggctgcttgccaatacggtgcggtatctgcagggcggcgggtcgtggcgggaggattggggacagctttcggggacggccgtgccgccccagggtgccgagccccagagcaacgcgggcccacgaccccatatcggggacacgttatttaccctgtttcgggcccccgagttgctggcccccaacggcgacctgtacaacgtgtttgcctgggccttggacgtcttggccaaacgcctccgtcccatgcacgtctttatcctggattacgaccaatcgcccgccggctgccgggacgccctgctgcaacttacctccgggatggtccagacccacgtcaccacccccggctccataccgacgatctgcgacctggcgcgcacgtttgcccgggagatgggggaggctaactga

SEQ ID NO: 10 - DNA, 1131 bp, synthetic construct
  source 1..1131: mol_type = other DNA
atggcttcgtacccctgccatcaacacgcgtctgcgttcgaccaggctgcgcgttctcgcggccatagcaaccgacgtacggcgttgcgccctcgccggcagcaagaagccacggaagtccgcctggagcagaaaatgcccacgctactgcgggtttatatagacggtcctcacgggatggggaaaaccaccaccacgcaactgctggtggccctgggttcgcgcgacgatatcgtctacgtacccgagccgatgacttactggcaggtgctgggggcttccgagacaatcgcgaacatctacaccacacaacaccgcctcgaccagggtgagatatcggccggggacgcggcggtggtaatgacaagcgcccagataacaatgggcatgccttatgccgtgaccgacgccgttctggctcctcatatcgggggggaggctgggagctcacatgccccgcccccggccctcaccctcatcttcgaccgccatcccatcgcccacctcctgtgctacccggccgcgcgataccttatgggcagcatgaccccccaggccgtgctggcgttcgtggccctcatcccgccgaccttgcccggcacaaacatcgtgttgggggcccttccggaggacagacacatcgaccgcctggccaaacgccagcgccccggcgagcggcttgacctggctatgctggccgcgattcgccgcgtttacgggctgcttgccaatacggtgcggtatctgcagggcggcgggtcgtggcgggaggattggggacagctttcggggacggccgtgccgccccagggtgccgagccccagagcaacgcgggcccacgaccccatatcggggacacgttatttaccctgtttcgggcccccgagttgctggcccccaacggcgacctgtacaacgtgtttgcctgggccttggacgtcttggccaaacgcctccgtcccatgcacgtctttatcctggattacgaccaatcgcccgccggctgccgggacgccctgctgcaacttacctccgggatggtccagacccacgtcaccacccccggctccataccgacgatctgcgacctggcgcgcacgtttgcccgggagatgggggaggctaactga

SEQ ID NO: 11 - DNA, 600 bp, synthetic construct
  source 1..600: mol_type = other DNA
atgaccgagtacaagcccacggtgcgcctcgccacccgcgacgacgtccctcgggccgtacgcaccctcgccgccgcgttcgccgactaccccgccacgcgccacaccgtggacccggaccgccacatcgagcgggtcaccgagctgcaagaactcttcctcacgcgcgtcgggctcgacatcggcaaggtgtgggtcgcggacgacggcgccgcggtggcggtctggaccacgccggagagcgtcgaagcgggggcggtgttcgccgagatcggcccgcgcatggccgagttgagcggttcccggctggccgcgcagcaacagatggaagggctcctggcgccgcaccggcccaaggagcccgcgtggttcctggccaccgtcggcgtctcgcccgaccaccagggcaagggtctgggcagcgccgtcgtgctccccggagtggaggcggccgagcgcgccggggtgcccgccttcctggagacctccgcgccccgcaacctccccttctacgagcggctcggcttcaccgtcaccgccgacgtcgaggtgcccgaaggaccgcgcacctggtgcatgacccgcaagcccggtgcctga

SEQ ID NO: 12 - DNA, 10 bp, synthetic construct
  source 1..10: mol_type = other DNA
gccaccatgg

SEQ ID NO: 13 - DNA, 666 bp, synthetic construct
  source 1..666: mol_type = other DNA
ggcgaaggcgatgggggtcttgaaggcgtgctggtactccacgatgcccagctcggtgttgctgtgcagctcctccacgcggcggaaggcgaacatggggcccccgttctgcaggatgctggggtggatggcgctcttgaagtgcatgtggctgtccaccacgaagctgtagtagccgccgtcgcgcaggctgaaggtgcgggcgaagctgcccaccagcacgttatcgcccatggggtgcaggtgctccacggtggcgttgctgcggatgatcttgtcggtgaagatcacgctgtcctcggggaagccggtgcccaccaccttgaagtcgccgatcacgcggccggcctcgtagcggtagctgaagctcacgtgcagcacgccgccgtcctcgtacttctcgatgcgggtgttggtgtagccgccgttgttgatggcgtgcaggaaggggttctcgtagccgctggggtaggtgccgaagtggtagaagccgtagcccatcacgtggctcagcaggtaggggctgaaggtcagggcgcctttggtgctcttcatcttgttggtcatgcggccctgctcgggggtgccctctccgccgcccaccagctcgaactccacgccgttcagggtgccggtgatgcggcactcgatcttcatggcgggcat

SEQ ID NO: 14 - DNA, 678 bp, synthetic construct
  source 1..678: mol_type = other DNA
atggcctcctccgaggacgtcatcaaggagttcatgcgcttcaaggtgcgcatggagggctccgtgaacggccacgagttcgagatcgagggcgagggcgagggccgcccctacgagggcacccagaccgccaagctgaaggtgaccaagggcggccccctgcccttcgcctgggacatcctgtcccctcagttccagtacggctccaaggcctacgtgaagcaccccgccgacatccccgactacttgaagctgtccttccccgagggcttcaagtgggagcgcgtgatgaacttcgaggacggcggcgtggtgaccgtgacccaggactcctccctgcaggacggcgagttcatctacaaggtgaagctgcgcggcaccaacttcccctccgacggccccgtaatgcagaagaagaccatgggctgggaggcctccaccgagcggatgtaccccgaggacggcgccctgaagggcgagatcaagatgaggctgaagctgaaggacggcggccactacgacgccgaggtcaagaccacctacatggccaagaagcccgtgcagctgcccggcgcctacaagaccgacatcaagctggacatcacctcccacaacgaggactacaccatcgtggaacagtacgagcgcgccgagggccgccactccaccggcgcctaa

SEQ ID NO: 15 - DNA, 181 bp, Human immunodeficiency virus 1
  source 1..181: mol_type = genomic DNA
gggtctctctggttagaccagatctgagcctgggagctctctggctaactagggaacccactgcttaagcctcaataaagcttgccttgagtgcttcaagtagtgtgtgcccgtctgttgtgtgactctggtaactagagatccctcagacccttttagtcagtgtggaaaatctctagca

SEQ ID NO: 16 - DNA, 126 bp, Human immunodeficiency virus 1
  source 1..126: mol_type = genomic DNA
ctctctcgacgcaggactcggcttgctgaagcgcgcacggcaagaggcgaggggcggcgactggtgagtacgccaaaaattttgactagcggaggctagaaggagagagatgggtgcgagagcgtc

SEQ ID NO: 17 - DNA, 234 bp, Human immunodeficiency virus 1
  source 1..234: mol_type = genomic DNA
aggagctttgttccttgggttcttgggagcagcaggaagcactatgggcgcagcgtcaatgacgctgacggtacaggccagacaattattgtctggtatagtgcagcagcagaacaatttgctgagggctattgaggcgcaacagcatctgttgcaactcacagtctggggcatcaagcagctccaagcaagaatcctagctgtggaaagatacctaaaggatcaacagctcct

SEQ ID NO: 18 - DNA, 588 bp, Woodchuck hepatitis virus
  source 1..588: mol_type = genomic DNA
aatcaacctctggattacaaaatttgtgaaagattgactggtattcttaactatgttgctccttttacgctatgtggatacgctgctttaatgcctttgtatcatgctattgcttcccgtatggctttcattttctcctccttgtataaatcctggttgctgtctctttatgaggagttgtggcccgttgtcaggcaacgtggcgtggtgtgcactgtgtttgctgacgcaacccccactggttggggcattgccaccacctgtcagctcctttccgggactttcgctttccccctccctattgccacggcggaactcatcgccgcctgccttgcccgctgctggacaggggctcggctgttgggcactgacaattccgtggtgttgtcggggaagctgacgtcctttccatggctgctcgcctgtgttgccacctggattctgcgcgggacgtccttctgctacgtcccttcggccctcaatccagcggaccttccttcccgcggcctgctgccggctctgcggcctcttccgcgtctcgccttcgccctcagacgagtcggatctccctttgggccgcctccccgc

SEQ ID NO: 19 - DNA, 36 bp, synthetic construct
  source 1..36: mol_type = other DNA
gcatggtggcggatccagctctgcttatataggcct

SEQ ID NO: 20 - DNA, 40 bp, synthetic construct
  source 1..40: mol_type = other DNA
tggggctcacctcgacatggtaatagcgatgactaatacg

SEQ ID NO: 21 - DNA, 18 bp, synthetic construct
  source 1..18: mol_type = other DNA
tcgaggtgagccccacgt

SEQ ID NO: 22 - DNA, 90 bp, synthetic construct
  source 1..90: mol_type = other DNA
ggagccctccatgcgcaccttgaagcgcatgaactccttgatgacgtcctcggaggaggccatggtggcctgtaggaaaaagaagaaggc

SEQ ID NO: 23 - DNA, 34 bp, synthetic construct
  source 1..34: mol_type = other DNA
gcatggtggcggatcccgaaaggcccggagatga

SEQ ID NO: 24 - DNA, 36 bp, synthetic construct
  source 1..36: mol_type = other DNA
atcgctattaccatggggtaggggaggcgcttttcc

SEQ ID NO: 25 - DNA, 25 bp, synthetic construct
  source 1..25: mol_type = other DNA
catggtaatagcgatgactaatacg

SEQ ID NO: 26 - DNA, 89 bp, synthetic construct
  source 1..89: mol_type = other DNA
ggagccctccatgcgcaccttgaagcgcatgaactccttgatgacgtcctcggaggaggccatggtggcagctctgcttatataggcct

SEQ ID NO: 27 - DNA, 40 bp, synthetic construct
  source 1..40: mol_type = other DNA
gcgcctcccctaccccatggtaatagcgatgactaatacg

SEQ ID NO: 28 - DNA, 21 bp, synthetic construct
  source 1..21: mol_type = other DNA
gggtaggggaggcgcttttcc

SEQ ID NO: 29 - DNA, 87 bp, synthetic construct
  source 1..87: mol_type = other DNA
ggagccctccatgcgcaccttgaagcgcatgaactccttgatgacgtcctcggaggaggccatggtggccgaaaggcccggagatga

SEQ ID NO: 30 - DNA, 31 bp, synthetic construct
  source 1..31: mol_type = other DNA
ctgtcatcgaattccaaatccctcggaagct

SEQ ID NO: 31 - DNA, 32 bp, synthetic construct
  source 1..32: mol_type = other DNA
taactcgagaacatcccacctcccctgcgagc

SEQ ID NO: 32 - DNA, 21 bp, synthetic construct
  source 1..21: mol_type = other DNA
gatgttctcgagttaggcgaa

SEQ ID NO: 33 - DNA, 18 bp, synthetic construct
  source 1..18: mol_type = other DNA
cgggctgcaggaattcac

SEQ ID NO: 34 - DNA, 33 bp, synthetic construct
  source 1..33: mol_type = other DNA
gcctgtcatcgaattcccacctcccctgcgagc

SEQ ID NO: 35 - DNA, 32 bp, synthetic construct
  source 1..32: mol_type = other DNA
taactcgagaacatccaaatccctcggaagct

SEQ ID NO: 36 - DNA, 31 bp, synthetic construct
  source 1..31: mol_type = other DNA
cgtctagagagtttccacctcccctgcgagc

SEQ ID NO: 37 - DNA, 37 bp, synthetic construct
  source 1..37: mol_type = other DNA
caccacgcgtgtttaacttgtttattgcagcttataa

SEQ ID NO: 38 - DNA, 31 bp, synthetic construct
  source 1..31: mol_type = other DNA
cgtctagagagtttcaaatccctcggaagct

SEQ ID NO: 39 - DNA, 17 bp, synthetic construct
  source 1..17: mol_type = other DNA
ccacctcccctgcgagc

SEQ ID NO: 40 - DNA, 41 bp, synthetic construct
  source 1..41: mol_type = other DNA
tcgcaggggaggtggagatccagacatgataagatacattg

SEQ ID NO: 41 - DNA, 33 bp, synthetic construct
  source 1..33: mol_type = other DNA
gcctgtcatcgaattccaaatccctcggaagct

SEQ ID NO: 42 - DNA, 33 bp, synthetic construct
  source 1..33: mol_type = other DNA
cgagaacatcgaattcccacctcccctgcgagc

SEQ ID NO: 43 - DNA, 33 bp, synthetic construct; identical to SEQ ID NO: 34
  source 1..33: mol_type = other DNA

SEQ ID NO: 44 - DNA, 33 bp, synthetic construct
  source 1..33: mol_type = other DNA
cgagaacatcgaattccaaatccctcggaagct

SEQ ID NO: 45 - DNA, 30 bp, synthetic construct
  source 1..30: mol_type = other DNA
accggtgccaccatggcttcgtacccctgc

SEQ ID NO: 46 - DNA, 26 bp, synthetic construct
  source 1..26: mol_type = other DNA
accggtctcagttagcctcccccatc

SEQ ID NO: 47 - DNA, 30 bp, synthetic construct
  source 1..30: mol_type = other DNA
cgccatcccatcgcccacctcctgtgctac

SEQ ID NO: 48 - DNA, 30 bp, synthetic construct
  source 1..30: mol_type = other DNA
gtagcacaggaggtgggcgatgggatggcg

SEQ ID NO: 49 - DNA, 32 bp, synthetic construct
  source 1..32: mol_type = other DNA
gctagctctagagagtttaaacacgcgtggtg

SEQ ID NO: 50 - DNA, 27 bp, synthetic construct
  source 1..27: mol_type = other DNA
tccggaccaaaaaagcctcctcactac

SEQ ID NO: 51 - DNA, 31 bp, synthetic construct
  source 1..31: mol_type = other DNA
ggtaccgcggggaggcggcccaaagggagat

SEQ ID NO: 52 - DNA, 23 bp, synthetic construct
  source 1..23: mol_type = other DNA
tgtacaacgtgtttgcctgggcc

SEQ ID NO: 53 - DNA, 37 bp, synthetic construct
  source 1..37: mol_type = other DNA
cgtcgacggttaacggggataccccctagagccccag